European Patent Application EP 4 324 910 A1, published February 21, 2024. Title: 一株耐盐芽孢杆菌及其应用. Applicant: 北京市农林科学院. Application CN. The sequence listing filed with the application follows.

SEQUENCE LISTING (2 sequences)

SEQ ID NO: 1 - DNA, 1446 bp, Bacillus halotolerans
  source 1..1446: mol_type = genomic DNA
ctagcgctgctatactgcaagtcgagcggacagatgggagcttgctccctgatgttagcggcggacgggtgagtaacacgtgggtaacctgcctgtaagactgggataactccgggaaaccggggctaataccggatgcttgtttgaaccgcatggttcaaacataaaaggtggcttcggctaccacttacagatggacccgcggcgcattagctagttggtgaggtaatggctcaccaaggcaacgatgcgtagccgacctgagagggtgatcggccacactgggactgagacacggcccagactcctacgggaggcagcagtagggaatcttccgcaatggacgaaagtctgacggagcaacgccgcgtgagtgatgaaggttttcggatcgtaaagctctgttgttagggaagaacaagtaccgttcgaatagggcggtaccttgacggtacctaaccagaaagccacggctaactacgtgccagcagccgcggtaatacgtaggtggcaagcgttgtccggaattattgggskwaaagggytcscaggcggttccttaagtytgawgkgaaagcccccggytcaaccggggagggtcattggaaactggggaacttgagtgcagaagaggagagtggaattccacgtgtagcggtgaaatgcgtagagatgtggaggaacaccagtggcgaaggcgactctctggtctgtaactgacgctgaggagcgaaagcgtggggagcgaacaggattagataccctggtagtccacgccgtaaacgatgagtgctaagtgttagggggtttccgccccttagtgctgcagctaacgcattaagcactccgcctggggartacggtcgcaagactgaaactcmaaggaattgacgggggcccgcacaagcggkgragcwtgkggtttawtycraagcamsgcgaagaaccttaccaggtcttgacatcctctgacaatcctagagataggacgtccccttcgggggcagagtgacaggtggtgcatggttgtcgtcagctcgtgtcgtgagatgttgggttaagtcccgcaacgagcgcaacccttgatcttagttgccagcattcagttgggcactctaaggtgactgccggtgacaaaccggaggaaggtggggatgacgtcaaatcatcatgccccttatgacctgggctacacacgtgctacaatggacagaacaaagggcagcgaaaccgcgaggttaagccaatcccacaaatctgttctcagttcggatcgcagtctgcaactcgactgcgtgaagctggaatcgctagtaatcgcggatcagcatgccgcggtgaatacgttcccgggccttgtacacaccgcccgtcacaccacgagagtttgtaacacccgaagtcggtgaggtaacctttatgagccagccgccgaagggaccccct

SEQ ID NO: 2 - DNA, 872 bp, Bacillus halotolerans
  source 1..872: mol_type = genomic DNA
ggtcgttacgcgttatcaacagagcttgatgtgactgttcaccgtgacggaaaaatccatcgccaagtctataaccgcggtgtcccggtttctgatcttgaggttattggcgaaacggatcatacaggaacgactacacactttgttccagatcctgaaatcttcacggaaacaactgagtatgaatatgatttgcttgctaaccgtgttcgcgaactagcctttttgacaaaaggcgtaaacatcacgattgaagataaacgtgaaggccaagagcgcaaaaatgagtatcattacgaaggcggaattaaaagctatgtagagtatttaaaccgctccaaagaagttgtccatgaagagccgatttatattgaaggcgaaaaggacggcattacggttgaagtcgctctgcaatacaatgacagctacacaagcaatatttactcatttacaaacaatatcaacacgtacgaaggcggtacccacgaagccggttttaaaacggggctgactcgtgtcatcaatgattacgccagaaaaaaaggactcataaaagaaaatgatccaaacttaagcggagatgatgtgagagaagggcttaccgcgattatctcgatcaaacacccggatccgcagttcgaaggccaaacgaaaacaaaactaggcaactcagaggcgcggacgatcacagatacgttattttctgctgcgttggaaacctttatgctggaaaatccagatgcggccaaaaaaatcgttgacaaaggcttaatggcagcaagagcaagaatggctgcgaaaaaagcgcgtgaattaacgcgccgcaaaagcgctttggagatttcaaaccttcctggtaaattagcggactg